European Patent Application EP 4 563 703 A1, published June 4, 2025. Title: Artificial receptor having shedding structure. Applicant: Kyoto University. The sequence listing filed with the application follows.

SEQUENCE LISTING (36 sequences)

SEQ ID NO: 1 - DNA, 978 bp, Mus musculus
  source 1..978: mol_type = genomic DNA
  CDS 1..978: note = Cleavable-TM domain of Notch; protein_id = 2; translation = ILDYSFTGGAGRDIPPPQIEEACELPECQVDAGNKVCNLQCNNHACGWDGGDCSLNFNDPWKNCTQSLQCWKYFSDGHCDSQCNSAGCLFDGFDCQLTEGQCNPLYDQYCKDHFSDGHCDQGCNSAECEWDGLDCAEHVPERLAAGTLVLVVLLPPDQLRNNSFHFLRELSHVLHTNVVFKRDAQGQQMIFPYYGHEEELRKHPIKRSTVGWATSSLLPGTSGGRQRRELDPMDIRGSIVYLEIDNRQCVQSSSQCFQSATDVAAFLGALASLGSLNIPYKIEAVKSEPVEPPLPSQLHLMYVAAAAFVLLFFVGCGVLLSRKRRR
atcctggactacagcttcacaggtggcgctgggcgcgacattcccccaccgcagattgaggaggcctgtgagctgcctgagtgccaggtggatgcaggcaataaggtctgcaacctgcagtgtaataatcacgcatgtggctgggatggtggcgactgctccctcaacttcaatgacccctggaagaactgcacgcagtctctacagtgctggaagtattttagcgacggccactgtgacagccagtgcaactcggccggctgcctctttgatggcttcgactgccagctcaccgagggacagtgcaaccccctgtatgaccagtactgcaaggaccacttcagtgatggccactgcgaccagggctgtaacagtgccgaatgtgagtgggatggcctagactgtgctgagcatgtacccgagcggctggcagccggcaccctggtgctggtggtgctgcttccacccgaccagctacggaacaactccttccactttctgcgggagctcagccacgtgctgcacaccaacgtggtcttcaagcgtgatgcgcaaggccagcagatgatcttcccgtactatggccacgaggaagagctgcgcaagcacccaatcaagcgctctacagtgggttgggccacctcttcactgcttcctggtaccagtggtgggcgccagcgcagggagctggaccccatggacatccgtggctccattgtctacctggagatcgacaaccggcaatgtgtgcagtcatcctcgcagtgcttccagagtgccaccgatgtggctgccttcctaggtgctcttgcgtcacttggcagcctcaatattccttacaagattgaggccgtgaagagtgagccggtggagcctccgctgccctcgcagctgcacctcatgtacgtggcagcggccgccttcgtgctcctgttctttgtgggctgtggggtgctgctgtcccgcaagcgccggcgg

SEQ ID NO: 2 - protein, 326 aa, Mus musculus
ILDYSFTGGAGRDIPPPQIEEACELPECQVDAGNKVCNLQCNNHACGWDGGDCSLNFNDPWKNCTQSLQCWKYFSDGHCDSQCNSAGCLFDGFDCQLTEGQCNPLYDQYCKDHFSDGHCDQGCNSAECEWDGLDCAEHVPERLAAGTLVLVVLLPPDQLRNNSFHFLRELSHVLHTNVVFKRDAQGQQMIFPYYGHEEELRKHPIKRSTVGWATSSLLPGTSGGRQRRELDPMDIRGSIVYLEIDNRQCVQSSSQCFQSATDVAAFLGALASLGSLNIPYKIEAVKSEPVEPPLPSQLHLMYVAAAAFVLLFFVGCGVLLSRKRRR

SEQ ID NO: 3 - DNA, 495 bp, Homo sapiens
  source 1..495: mol_type = genomic DNA
  CDS 1..495: note = Cleavable-TM domain of APP; protein_id = 4; translation = QDEVDELLQKEQNYSDDVLANMISEPRISYGNDALMPSLTETKTTVELLPVNGEFSLDDLQPWHSFGADSVPANTENEVEPVDARPAADRGLTTRPGSGLTNIKTEEISEVKMDAEFRHDSGYEVHHQKLVFFAEDVGSNKGAIIGLMVGGVVIATVIVITLVML
caggatgaagttgatgagctgcttcagaaagagcaaaactattcagatgacgtcttggccaacatgattagtgaaccaaggatcagttacggaaacgatgctctcatgccatctttgaccgaaacgaaaaccaccgtggagctccttcccgtgaatggagagttcagcctggacgatctccagccgtggcattcttttggggctgactctgtgccagccaacacagaaaacgaagttgagcctgttgatgcccgccctgctgccgaccgaggactgaccactcgaccaggttctgggttgacaaatatcaagacggaggagatctctgaagtgaaaatggatgcagaattccgacatgactcaggatatgaagttcatcatcaaaaattggtgttctttgcagaagatgtgggttcaaacaaaggtgcaatcattggactcatggtgggcggtgttgtcatagcgacagtgatcgtcatcaccttggtgatgctg

SEQ ID NO: 4 - protein, 165 aa, Homo sapiens
QDEVDELLQKEQNYSDDVLANMISEPRISYGNDALMPSLTETKTTVELLPVNGEFSLDDLQPWHSFGADSVPANTENEVEPVDARPAADRGLTTRPGSGLTNIKTEEISEVKMDAEFRHDSGYEVHHQKLVFFAEDVGSNKGAIIGLMVGGVVIATVIVITLVML

SEQ ID NO: 5 - DNA, 249 bp, Homo sapiens
  source 1..249: mol_type = genomic DNA
  CDS 1..249: note = CD8-TM domain; protein_id = 6; translation = FVPVFLPAKPTTTPAPRPPTPAPTIASQPLSLRPEACRPAAGGAVHTRGLDFACDIYIWAPLAGTCGVLLLSLVITLYCNHRN
tttgtgcccgtgtttctgcctgccaaaccaaccaccaccccagccccaagaccaccaacacctgcccctacaatcgcctcacagccactgagcctgagaccagaggcctgtagaccagccgccggaggagccgtgcatacaagaggcctggattttgcctgcgacatctacatctgggccccactggccggcacatgtggagtgctgctgctgtctctggtgatcaccctgtactgcaaccacagaaac

SEQ ID NO: 6 - protein, 83 aa, Homo sapiens
FVPVFLPAKPTTTPAPRPPTPAPTIASQPLSLRPEACRPAAGGAVHTRGLDFACDIYIWAPLAGTCGVLLLSLVITLYCNHRN

SEQ ID NO: 7 - DNA, 495 bp, Homo sapiens
  source 1..495: mol_type = genomic DNA
  CDS 1..495: note = Cleavable-TM domain of APP mutant; protein_id = 8; translation = QDEVDELLQKEQNYSDDVLANMISEPRISYGNDALMPSLTETKTTVELLPVNGEFSLDDLQPWHSFGADSVPANTENEVEPVDARPAADRGLTTRPGSGLTNIKTEEISEVNLDAEFRHDSGYEVHHQKLVFFAEDVGSNKGAIIGLMVGGVVIATVIVITLVML
caggatgaagttgatgagctgcttcagaaagagcaaaactattcagatgacgtcttggccaacatgattagtgaaccaaggatcagttacggaaacgatgctctcatgccatctttgaccgaaacgaaaaccaccgtggagctccttcccgtgaatggagagttcagcctggacgatctccagccgtggcattcttttggggctgactctgtgccagccaacacagaaaacgaagttgagcctgttgatgcccgccctgctgccgaccgaggactgaccactcgaccaggttctgggttgacaaatatcaagacggaggagatctctgaagtgaatctggatgcagaattccgacatgactcaggatatgaagttcatcatcaaaaattggtgttctttgcagaagatgtgggttcaaacaaaggtgcaatcattggactcatggtgggcggtgttgtcatagcgacagtgatcgtcatcaccttggtgatgctg

SEQ ID NO: 8 - protein, 165 aa, Homo sapiens
QDEVDELLQKEQNYSDDVLANMISEPRISYGNDALMPSLTETKTTVELLPVNGEFSLDDLQPWHSFGADSVPANTENEVEPVDARPAADRGLTTRPGSGLTNIKTEEISEVNLDAEFRHDSGYEVHHQKLVFFAEDVGSNKGAIIGLMVGGVVIATVIVITLVML

SEQ ID NO: 9 - DNA, 336 bp, Homo sapiens
  source 1..336: mol_type = genomic DNA
  CDS 1..336: note = signaling domain of CD3 zeta; protein_id = 10; translation = RVKFSRSADAPAYQQGQNQLYNELNLGRREEYDVLDKRRGRDPEMGGKPRRKNPQEGLYNELQKDKMAEAYSEIGMKGERRRGKGHDGLYQGLSTATKDTYDALHMQALPPR
agagtgaagttcagcagaagcgccgatgccccagcctaccagcagggccagaaccagctgtataacgagctgaacctgggcagaagagaggagtacgacgtgctggacaagagaagaggcagagaccccgagatgggcggcaagcccagaagaaagaacccccaggagggcctgtacaatgaacttcagaaggacaagatggccgaggcctacagcgagatcggcatgaagggcgagagaagaagaggcaagggccacgatggcctgtaccagggactgagcaccgccaccaaggatacctacgacgccctgcacatgcaagctctgcctccaaga

SEQ ID NO: 10 - protein, 112 aa, Homo sapiens
RVKFSRSADAPAYQQGQNQLYNELNLGRREEYDVLDKRRGRDPEMGGKPRRKNPQEGLYNELQKDKMAEAYSEIGMKGERRRGKGHDGLYQGLSTATKDTYDALHMQALPPR

SEQ ID NO: 11 - DNA, 123 bp, Homo sapiens
  source 1..123: mol_type = genomic DNA
  CDS 1..123: note = signaling domain of CD28; protein_id = 12; translation = RSKRSRLLHSDYMNMTPRRPGPTRKHYQPYAPPRDFAAYRS
agaagcaagagaagcagactgctgcacagcgactacatgaacatgacccccagaagacccggccccaccagaaaacactaccagccctacgcccctcccagagacttcgccgcctacagaagc

SEQ ID NO: 12 - protein, 41 aa, Homo sapiens
RSKRSRLLHSDYMNMTPRRPGPTRKHYQPYAPPRDFAAYRS

SEQ ID NO: 13 - DNA, 141 bp, Homo sapiens
  source 1..141: mol_type = genomic DNA
  CDS 1..141: note = signaling domain of 4-1BB; protein_id = 14; translation = RFSVVKRGRKKLLYIFKQPFMRPVQTTQEEDGCSCRFPEEEEGGCEL
agattcagcgtggtgaagagaggcagaaagaagctgctgtacatcttcaagcagcccttcatgagacccgtgcagaccacccaggaggaggacggctgcagctgcagattcccagaagaggaggagggcggctgtgagctg

SEQ ID NO: 14 - protein, 47 aa, Homo sapiens
RFSVVKRGRKKLLYIFKQPFMRPVQTTQEEDGCSCRFPEEEEGGCEL

SEQ ID NO: 15 - DNA, 801 bp, Homo sapiens
  source 1..801: mol_type = genomic DNA
  CDS 1..801: note = FCM63 CD19-specific scFv; protein_id = 16; translation = MLLLVTSLLLCELPHPAFLLIPDIQMTQTTSSLSASLGDRVTISCRASQDISKYLNWYQQKPDGTVKLLIYHTSRLHSGVPSRFSGSGSGTDYSLTISNLEQEDIATYFCQQGNTLPYTFGGGTKLEITGSTSGSGKPGSGEGSTKGEVKLQESGPGLVAPSQSLSVTCTVSGVSLPDYGVSWIRQPPRKGLEWLGVIWGSETTYYNSALKSRLTIIKDNSKSQVFLKMNSLQTDDTAIYYCAKHYYYGGSYAMDYWGQGTSVTVSS
atgctgctgctggtgaccagcctgctgctgtgtgagctgcctcaccccgcctttctgctgatccctgacatccagatgacccagactaccagcagcctgagcgcctctctgggcgatagagtgaccatcagctgcagagccagccaggacatcagcaagtacctgaactggtaccagcagaagcccgacggcaccgtgaagctgctgatctaccacaccagcagactgcacagcggcgtgcccagcagatttagcggaagcggcagcggcaccgattacagcctgaccatcagcaacctggagcaggaggacatcgccacctacttctgccagcagggcaacaccctgccatacacattcggcggcggcacaaagctggagatcaccggcagcacaagcggaagcggcaaaccaggaagcggcgagggctctacaaagggcgaggtgaaactgcaggaaagcggaccaggcctggtggccccttctcagagcctgtctgtgacctgtacagtgagcggcgtgagcctgccagactatggcgtgagctggatcagacagccccccagaaagggcctggaatggctgggagtgatctggggcagcgagacaacctactacaacagcgccctgaagagcagactgaccattattaaggacaacagcaagagccaggtgttcctgaagatgaacagcctgcagaccgacgacaccgccatctactactgcgccaagcactactactacggcggcagctacgccatggattactggggccagggcacaagcgtgaccgtgagctct

SEQ ID NO: 16 - protein, 267 aa, Homo sapiens
MLLLVTSLLLCELPHPAFLLIPDIQMTQTTSSLSASLGDRVTISCRASQDISKYLNWYQQKPDGTVKLLIYHTSRLHSGVPSRFSGSGSGTDYSLTISNLEQEDIATYFCQQGNTLPYTFGGGTKLEITGSTSGSGKPGSGEGSTKGEVKLQESGPGLVAPSQSLSVTCTVSGVSLPDYGVSWIRQPPRKGLEWLGVIWGSETTYYNSALKSRLTIIKDNSKSQVFLKMNSLQTDDTAIYYCAKHYYYGGSYAMDYWGQGTSVTVSS

SEQ ID NO: 17 - DNA, 36 bp, Homo sapiens
  source 1..36: mol_type = genomic DNA
  CDS 1..36: note = hinge domain of IgG4; protein_id = 18; translation = ESKYGPPCPPCP
gagtctaagtacggcccaccctgccctccctgcccc

SEQ ID NO: 18 - protein, 12 aa, Homo sapiens
ESKYGPPCPPCP

SEQ ID NO: 19 - DNA, 720 bp, synthetic construct
  source 1..720: mol_type = other DNA
  CDS 1..720: note = EGFP; protein_id = 20; translation = MVSKGEELFTGVVPILVELDGDVNGHKFSVSGEGEGDATYGKLTLKFICTTGKLPVPWPTLVTTLTYGVQCFSRYPDHMKQHDFFKSAMPEGYVQERTIFFKDDGNYKTRAEVKFEGDTLVNRIELKGIDFKEDGNILGHKLEYNYNSHNVYIMADKQKNGIKVNFKIRHNIEDGSVQLADHYQQNTPIGDGPVLLPDNHYLSTQSALSKDPNEKRDHMVLLEFVTAAGITLGMDELYK
atggtgagcaagggcgaggagctgttcaccggggtggtgcccatcctggtcgagctggacggcgacgtaaacggccacaagttcagcgtgtccggcgagggcgagggcgatgccacctacggcaagctgaccctgaagttcatctgcaccaccggcaagctgcccgtgccctggcccaccctcgtgaccaccctgacctacggcgtgcagtgcttcagccgctaccccgaccacatgaagcagcacgacttcttcaagtccgccatgcccgaaggctacgtccaggagcgcaccatcttcttcaaggacgacggcaactacaagacccgcgccgaggtgaagttcgagggcgacaccctggtgaaccgcatcgagctgaagggcatcgacttcaaggaggacggcaacatcctggggcacaagctggagtacaactacaacagccacaacgtctatatcatggccgacaagcagaagaacggcatcaaggtgaacttcaagatccgccacaacatcgaggacggcagcgtgcagctcgccgaccactaccagcagaacacccccatcggcgacggccccgtgctgctgcccgacaaccactacctgagcacccagtccgccctgagcaaagaccccaacgagaagcgcgatcacatggtcctgctggagttcgtgaccgccgccgggatcactctcggcatggacgagctgtacaagtaa

SEQ ID NO: 20 - protein, 239 aa, synthetic construct
  REGION 1..239: note = Synthetic Construct
MVSKGEELFTGVVPILVELDGDVNGHKFSVSGEGEGDATYGKLTLKFICTTGKLPVPWPTLVTTLTYGVQCFSRYPDHMKQHDFFKSAMPEGYVQERTIFFKDDGNYKTRAEVKFEGDTLVNRIELKGIDFKEDGNILGHKLEYNYNSHNVYIMADKQKNGIKVNFKIRHNIEDGSVQLADHYQQNTPIGDGPVLLPDNHYLSTQSALSKDPNEKRDHMVLLEFVTAAGITLGMDELYK

SEQ ID NO: 21 - DNA, 117 bp, Homo sapiens
  source 1..117: mol_type = genomic DNA
  CDS 1..117: note = Cleavable-TM domain of CD28; protein_id = 22; translation = CPSPLFPGPSKPFWVLVVVGGVLACYSLLVTVAFIIFWV
tgtccaagtcccctatttcccggaccttctaagcccttttgggtgctggtggtggttggtggagtcctggcttgctatagcttgctagtaacagtggcctttattattttctgggtg

SEQ ID NO: 22 - protein, 39 aa, Homo sapiens
CPSPLFPGPSKPFWVLVVVGGVLACYSLLVTVAFIIFWV

SEQ ID NO: 23 - DNA, 90 bp, Homo sapiens
  source 1..90: mol_type = genomic DNA
  CDS 1..90: note = hinge domain of CD28; protein_id = 24; translation = LDNEKSNGTIIHVKGKHLCPSPLFPGPSKP
cttgataatgaaaagtcaaacggaacaatcattcacgtgaagggcaagcacctctgtccgtcacccttgttccctggtccatccaagcca

SEQ ID NO: 24 - protein, 30 aa, Homo sapiens
LDNEKSNGTIIHVKGKHLCPSPLFPGPSKP

SEQ ID NO: 25 - DNA, 36 bp, Homo sapiens
  source 1..36: mol_type = genomic DNA
  CDS 1..36: note = hinge domain of CD28; protein_id = 26; translation = CPSPLFPGPSKP
tgtccaagtcccctatttcccggaccttctaagccc

SEQ ID NO: 26 - protein, 12 aa, Homo sapiens
CPSPLFPGPSKP

SEQ ID NO: 27 - DNA, 1008 bp, Homo sapiens
  source 1..1008: mol_type = genomic DNA
  CDS 1..1008: note = hCleavable-TM domain of Notch; protein_id = 28; translation = ILDYSFGGGAGRDIPPPLIEEACELPECQEDAGNKVCSLQCNNHACGWDGGDCSLNFNDPWKNCTQSLQCWKYFSDGHCDSQCNSAGCLFDGFDCQRAEGQCNPLYDQYCKDHFSDGHCDQGCNSAECEWDGLDCAEHVPERLAAGTLVVVVLMPPEQLRNSSFHFLRELSRVLHTNVVFKRDAHGQQMIFPYYGREEELRKHPIKRAAEGWAAPDALLGQVKASLLPGGSEGGRRRRELDPMDVRGSIVYLEIDNRQCVQASSQCFQSATDVAAFLGALASLGSLNIPYKIEAVQSETVEPPPPAQLHFMYVAAAAFVLLFFVGCGVLLSRKRRR
atcctggactacagcttcgggggtggggccgggcgcgacatccccccgccgctgatcgaggaggcgtgcgagctgcccgagtgccaggaggacgcgggcaacaaggtctgcagcctgcagtgcaacaaccacgcgtgcggctgggacggcggtgactgctccctcaacttcaatgacccctggaagaactgcacgcagtctctgcagtgctggaagtacttcagtgacggccactgtgacagccagtgcaactcagccggctgcctcttcgacggctttgactgccagcgtgcggaaggccagtgcaaccccctgtacgaccagtactgcaaggaccacttcagcgacgggcactgcgaccagggctgcaacagcgcggagtgcgagtgggacgggctggactgtgcggagcatgtacccgagaggctggcggccggcacgctggtggtggtggtgctgatgccgccggagcagctgcgcaacagctccttccacttcctgcgggagctcagccgcgtgctgcacaccaacgtggtcttcaagcgtgacgcacacggccagcagatgatcttcccctactacggccgcgaggaggagctgcgcaagcaccccatcaagcgtgccgccgagggctgggccgcacctgacgccctgctgggccaggtgaaggcctcgctgctccctggtggcagcgagggtgggcggcggcggagggagctggaccccatggacgtccgcggctccatcgtctacctggagattgacaaccggcagtgtgtgcaggcctcctcgcagtgcttccagagtgccaccgacgtggccgcattcctgggagcgctcgcctcgctgggcagcctcaacatcccctacaagatcgaggccgtgcagagtgagaccgtggagccgcccccgccggcgcagctgcacttcatgtacgtggcggcggccgcctttgtgcttctgttcttcgtgggctgcggggtgctgctgtcccgcaagcgccggcgg

SEQ ID NO: 28 - protein, 336 aa, Homo sapiens
ILDYSFGGGAGRDIPPPLIEEACELPECQEDAGNKVCSLQCNNHACGWDGGDCSLNFNDPWKNCTQSLQCWKYFSDGHCDSQCNSAGCLFDGFDCQRAEGQCNPLYDQYCKDHFSDGHCDQGCNSAECEWDGLDCAEHVPERLAAGTLVVVVLMPPEQLRNSSFHFLRELSRVLHTNVVFKRDAHGQQMIFPYYGREEELRKHPIKRAAEGWAAPDALLGQVKASLLPGGSEGGRRRRELDPMDVRGSIVYLEIDNRQCVQASSQCFQSATDVAAFLGALASLGSLNIPYKIEAVQSETVEPPPPAQLHFMYVAAAAFVLLFFVGCGVLLSRKRRR

SEQ ID NO: 29 - DNA, 789 bp, synthetic construct
  source 1..789: mol_type = other DNA
  misc_feature 1..789: note = aTRBV12-specific ScFv
  CDS 1..789: protein_id = 30; translation = MLLLVTSLLLCELPHPAFLLIPENVLTQSPAIMSASLGEKVTMSCRASSSVNYIYWYQQKSDASPKLWIYYTSNLAPGVPTRFSGSGSGNSYSLTISSMEGEDAATYYCQQFTSSPFTFGQGTKLEIKGSTSGSGKPGSGEGSTKGDVQLVESGGGLVQPGGSRKLSCAASGFTFSNFGMHWVRQAPGKGLEWVAYISSGSSTIYYADTLKGRFTISRDNPKNTLFLQMTSLRSEDTAMYYCARRGEGAMDYWGQGTSVTVSS
atgctgctgctggtgaccagcctgctgctgtgtgagctgcctcaccccgcctttctgctgatccctgaaaacgtgctgacccagagcccggcgattatgagcgcgagcctgggcgaaaaagtgaccatgagctgccgcgcgagcagcagcgtgaactatatttattggtatcagcagaaaagcgatgcgagcccgaaactgtggatttattataccagcaacctggcgccgggcgtgccgacccgctttagcggcagcggcagcggcaacagctatagcctgaccattagcagcatggaaggcgaagatgcggcgacctattattgccagcagtttaccagcagcccgtttacctttggccagggcaccaaactggaaattaaaggcagcacaagcggaagcggcaaaccaggaagcggcgagggctctacaaagggcgatgtgcagctggtggaaagcggcggcggcctggtgcagccgggcggcagccgcaaactgagctgcgcggcgagcggctttacctttagcaactttggcatgcattgggtgcgccaggcgccgggcaaaggcctggaatgggtggcgtatattagcagcggcagcagcaccatttattatgcggataccctgaaaggccgctttaccattagccgcgataacccgaaaaacaccctgtttctgcagatgaccagcctgcgcagcgaagataccgcgatgtattattgcgcgcgccgcggcgaaggcgcgatggattattggggccagggcaccagcgtgaccgtgagcagc

SEQ ID NO: 30 - protein, 263 aa, synthetic construct
MLLLVTSLLLCELPHPAFLLIPENVLTQSPAIMSASLGEKVTMSCRASSSVNYIYWYQQKSDASPKLWIYYTSNLAPGVPTRFSGSGSGNSYSLTISSMEGEDAATYYCQQFTSSPFTFGQGTKLEIKGSTSGSGKPGSGEGSTKGDVQLVESGGGLVQPGGSRKLSCAASGFTFSNFGMHWVRQAPGKGLEWVAYISSGSSTIYYADTLKGRFTISRDNPKNTLFLQMTSLRSEDTAMYYCARRGEGAMDYWGQGTSVTVSS

SEQ ID NO: 31 - DNA, 801 bp, synthetic construct
  source 1..801: mol_type = other DNA
  misc_feature 1..801: note = Her2-specific ScFV
  CDS 1..801: protein_id = 32; translation = MLLLVTSLLLCELPHPAFLLIPDIQMTQSPSSLSASVGDRVTITCRASQDVNTAVAWYQQKPGKAPKLLIYSASFLYSGVPSRFSGSRSGTDFTLTISSLQPEDFATYYCQQHYTTPPTFGQGTKVEIKGSTSGGGSGGGSGGGGSSEVQLVESGGGLVQPGGSLRLSCAASGFNIKDTYIHWVRQAPGKGLEWVARIYPTNGYTRYADSVKGRFTISADTSKNTAYLQMNSLRAEDTAVYYCSRWGGDGFYAMDYWGQGTLVTVSS
atgctcctgctggtgaccagcctcctgctgtgcgagctgccccaccccgcctttctgctgattcccgacatccagatgacccagtccccttcatctctctccgcctctgtgggagatagagtgaccatcacctgccgcgccagccaggacgtgaacactgccgtggcctggtaccagcagaagcccggcaaagccccaaagctgctgatttacagcgccagctttctgtacagcggcgtgccaagcaggttctccggctctagaagcggcaccgatttcaccctgaccatcagctctctgcagcccgaggattttgccacttactactgccagcagcattatacaacccctcccacttttggtcagggaaccaaggtcgaaatcaagggaagcacctccggcggcggaagcgggggggggtccggcggaggcggatcctctgaggtgcagctggtcgagagcggcgggggcctggtgcagcctggcggaagcctgagactgagttgcgcagctagcggcttcaacatcaaggacacatacattcactgggtgagacaggccccaggaaagggcctggagtgggtggcaagaatctatcccaccaatggctatacaaggtacgccgactccgtgaagggtaggtttaccatctccgccgacacctctaagaacactgcctacctgcagatgaattctctgagggccgaggataccgctgtgtattactgcagcagatggggcggcgatggcttctacgccatggactattgggggcagggcactctggtgaccgtgtcttcc

SEQ ID NO: 32 - protein, 267 aa, synthetic construct
MLLLVTSLLLCELPHPAFLLIPDIQMTQSPSSLSASVGDRVTITCRASQDVNTAVAWYQQKPGKAPKLLIYSASFLYSGVPSRFSGSRSGTDFTLTISSLQPEDFATYYCQQHYTTPPTFGQGTKVEIKGSTSGGGSGGGSGGGGSSEVQLVESGGGLVQPGGSLRLSCAASGFNIKDTYIHWVRQAPGKGLEWVARIYPTNGYTRYADSVKGRFTISADTSKNTAYLQMNSLRAEDTAVYYCSRWGGDGFYAMDYWGQGTLVTVSS

SEQ ID NO: 33 - protein, 316 aa, Homo sapiens
EACELPECQEDAGNKVCSLQCNNHACGWDGGDCSLNFNDPWKNCTQSLQCWKYFSDGHCDSQCNSAGCLFDGFDCQRAEGQCNPLYDQYCKDHFSDGHCDQGCNSAECEWDGLDCAEHVPERLAAGTLVVVVLMPPEQLRNSSFHFLRELSRVLHTNVVFKRDAHGQQMIFPYYGREEELRKHPIKRAAEGWAAPDALLGQVKASLLPGGSEGGRRRRELDPMDVRGSIVYLEIDNRQCVQASSQCFQSATDVAAFLGALASLGSLNIPYKIEAVQSETVEPPPPAQLHFMYVAAAAFVLLFFVGCGVLLSRKRRR

SEQ ID NO: 34 - protein, 275 aa, Homo sapiens
KNCTQSLQCWKYFSDGHCDSQCNSAGCLFDGFDCQRAEGQCNPLYDQYCKDHFSDGHCDQGCNSAECEWDGLDCAEHVPERLAAGTLVVVVLMPPEQLRNSSFHFLRELSRVLHTNVVFKRDAHGQQMIFPYYGREEELRKHPIKRAAEGWAAPDALLGQVKASLLPGGSEGGRRRRELDPMDVRGSIVYLEIDNRQCVQASSQCFQSATDVAAFLGALASLGSLNIPYKIEAVQSETVEPPPPAQLHFMYVAAAAFVLLFFVGCGVLLSRKRRR

SEQ ID NO: 35 - protein, 233 aa, Homo sapiens
PLYDQYCKDHFSDGHCDQGCNSAECEWDGLDCAEHVPERLAAGTLVVVVLMPPEQLRNSSFHFLRELSRVLHTNVVFKRDAHGQQMIFPYYGREEELRKHPIKRAAEGWAAPDALLGQVKASLLPGGSEGGRRRRELDPMDVRGSIVYLEIDNRQCVQASSQCFQSATDVAAFLGALASLGSLNIPYKIEAVQSETVEPPPPAQLHFMYVAAAAFVLLFFVGCGVLLSRKRRR

SEQ ID NO: 36 - protein, 203 aa, Homo sapiens
DCAEHVPERLAAGTLVVVVLMPPEQLRNSSFHFLRELSRVLHTNVVFKRDAHGQQMIFPYYGREEELRKHPIKRAAEGWAAPDALLGQVKASLLPGGSEGGRRRRELDPMDVRGSIVYLEIDNRQCVQASSQCFQSATDVAAFLGALASLGSLNIPYKIEAVQSETVEPPPPAQLHFMYVAAAAFVLLFFVGCGVLLSRKRRR